European Patent Application EP 4 782 541 A1, published July 29, 2026. Title: 靶向人源ROR1和CD3的双特异性抗体. Applicant: 南京蓬勃生物科技有限公司. The sequence listing filed with the application follows.

SEQUENCE LISTING (50 sequences)

SEQ ID NO: 1 - protein, 338 aa, synthetic construct
EVQLVESGGGLVQPGGSLRLSCAASGFISRFYAMGWYRQAPGKQRELVARISSMGWTYYADSVKGRFTISIDNSKNTLYLQMNSLRAEDTAVYYCNARNLWGQGTLVTVSSDKTHTCPPCPAPESTRGPSVFLFPPKPKDTLMISRTPEVTCVVVDVSHEDPEVKFNWYVDGVEVHNAKTKPREEQYNSTYRVVSVLTVLHQDWLNGKEYKCKVSNKALPAPIEKTISKAKGQPREPQVCTLPPSRDELTKNQVSLSCAVKGFYPSDIAVEWESNGQPENNYKTTPPVLDSDGSFFLVSKLTVDKSRWQQGNVFSCSVMHEALHNHYTQKSLSLSPGK

SEQ ID NO: 2 - protein, 455 aa, synthetic construct
EVQLVESGGGLVQPGRSLRLSCAASGFTFNTYAMNWVRQAPGKGLEWVARIRSKYNNYATYYADSVKDRFTISRDDSKSIAYLQMNSLKTEDTAVYYCVRHGNFGNSYVSWFAYWGQGTLVTVSSASTKGPSVFPLAPSSKSTSGGTAALGCLVKDYFPEPVTVSWNSGALTSGVHTFPAVLQSSGLYSLSSVVTVPSSSLGTQTYICNVNHKPSNTKVDKKVEPKSCDKTHTCPPCPAPESTRGPSVFLFPPKPKDTLMISRTPEVTCVVVDVSHEDPEVKFNWYVDGVEVHNAKTKPREEQYNSTYRVVSVLTVLHQDWLNGKEYKCKVSNKALPAPIEKTISKAKGQPREPQVYTLPPCRDELTKNQVSLWCLVKGFYPSDIAVEWESNGQPENNYKTTPPVLDSDGSFFLYSKLTVDKSRWQQGNVFSCSVMHEALHNHYTQKSLSLSPGK

SEQ ID NO: 3 - protein, 215 aa, synthetic construct
QTVVTQEPSLTVSPGGTVTLTCRSSTGAVTTSNYANWVQQKPGQAPRGLIGGTNKRAPGVPARFSGSLLGGKAALTLSGVQPEDEAEYFCALWYSNLWVFGGGTKLTVLGQPKAAPSVTLFPPSSEELQANKATLVCLISDFYPGAVTVAWKADSSPVKAGVETTTPSKQSNNKYAASSYLSLTPEQWKSHRSYSCQVTHEGSTVEKTVAPTECS

SEQ ID NO: 4 - protein, 338 aa, synthetic construct
EVQLVESGGGLVQPGGSLRLSCAASYFISRFYAVGWYRQAPGKQRELVARISSGGWTYYADSVKGRFTISIDNSKNTLYLQMNSLRAEDTAVYYCNARNLWGQGTLVTVSSDKTHTCPPCPAPESTRGPSVFLFPPKPKDTLMISRTPEVTCVVVDVSHEDPEVKFNWYVDGVEVHNAKTKPREEQYNSTYRVVSVLTVLHQDWLNGKEYKCKVSNKALPAPIEKTISKAKGQPREPQVCTLPPSRDELTKNQVSLSCAVKGFYPSDIAVEWESNGQPENNYKTTPPVLDSDGSFFLVSKLTVDKSRWQQGNVFSCSVMHEALHNHYTQKSLSLSPGK

SEQ ID NO: 5 - protein, 338 aa, synthetic construct
QVQLVESGGGVVQPGGSLRLSCAASGFVLRVNTVSWYRQAPGKQRELVALITSESNEYYDDSVKGRFTISRDNAKNTIYLHMNSLKPEDTGVYFCNFITTWGQGTQVTVSSDKTHTCPPCPAPESTRGPSVFLFPPKPKDTLMISRTPEVTCVVVDVSHEDPEVKFNWYVDGVEVHNAKTKPREEQYNSTYRVVSVLTVLHQDWLNGKEYKCKVSNKALPAPIEKTISKAKGQPREPQVCTLPPSRDELTKNQVSLSCAVKGFYPSDIAVEWESNGQPENNYKTTPPVLDSDGSFFLVSKLTVDKSRWQQGNVFSCSVMHEALHNHYTQKSLSLSPGK

SEQ ID NO: 6 - protein, 347 aa, synthetic construct
EVQLVESGGGLVQPGGSLRLSCAASGRSFSSFQMGWFRQAPGKEREFVAASGWSGGPTYYWDSVIGRFTISTDNSKNTLYLQMNSLRAEDTAVYYCYEDRVLSGRPVRYWGQGTLVTVSSDKTHTCPPCPAPESTRGPSVFLFPPKPKDTLMISRTPEVTCVVVDVSHEDPEVKFNWYVDGVEVHNAKTKPREEQYNSTYRVVSVLTVLHQDWLNGKEYKCKVSNKALPAPIEKTISKAKGQPREPQVCTLPPSRDELTKNQVSLSCAVKGFYPSDIAVEWESNGQPENNYKTTPPVLDSDGSFFLVSKLTVDKSRWQQGNVFSCSVMHEALHNHYTQKSLSLSPGK

SEQ ID NO: 7 - protein, 347 aa, synthetic construct
EVQLVESGGGLVQPGGSLRLSCAASGRSFSSFQMGWFRQAPGKEREFVAASGWSGGPTYYWDSVIGRFTISTDNSKNTLYLQMNSLRAEDTAVYYCYEDRVLSGRHVRYWGQGTLVTVSSDKTHTCPPCPAPESTRGPSVFLFPPKPKDTLMISRTPEVTCVVVDVSHEDPEVKFNWYVDGVEVHNAKTKPREEQYNSTYRVVSVLTVLHQDWLNGKEYKCKVSNKALPAPIEKTISKAKGQPREPQVCTLPPSRDELTKNQVSLSCAVKGFYPSDIAVEWESNGQPENNYKTTPPVLDSDGSFFLVSKLTVDKSRWQQGNVFSCSVMHEALHNHYTQKSLSLSPGK

SEQ ID NO: 8 - protein, 464 aa, synthetic construct
EVQLVESGGGLVQPGGSLRLSCAASGFISRFYAMGWYRQAPGKQRELVARISSMGWTYYADSVKGRFTISIDNSKNTLYLQMNSLRAEDTAVYYCNARNLWGQGTLVTVSSGGGGSGGGGSGGGGSEVQLVESGGGLVQPGGSLRLSCAASGFISRFYAMGWYRQAPGKQRELVARISSMGWTYYADSVKGRFTISIDNSKNTLYLQMNSLRAEDTAVYYCNARNLWGQGTLVTVSSDKTHTCPPCPAPESTRGPSVFLFPPKPKDTLMISRTPEVTCVVVDVSHEDPEVKFNWYVDGVEVHNAKTKPREEQYNSTYRVVSVLTVLHQDWLNGKEYKCKVSNKALPAPIEKTISKAKGQPREPQVCTLPPSRDELTKNQVSLSCAVKGFYPSDIAVEWESNGQPENNYKTTPPVLDSDGSFFLVSKLTVDKSRWQQGNVFSCSVMHEALHNHYTQKSLSLSPGK

SEQ ID NO: 9 - protein, 464 aa, synthetic construct
EVQLVESGGGLVQPGGSLRLSCAASYFISRFYAVGWYRQAPGKQRELVARISSGGWTYYADSVKGRFTISIDNSKNTLYLQMNSLRAEDTAVYYCNARNLWGQGTLVTVSSGGGGSGGGGSGGGGSEVQLVESGGGLVQPGGSLRLSCAASYFISRFYAVGWYRQAPGKQRELVARISSGGWTYYADSVKGRFTISIDNSKNTLYLQMNSLRAEDTAVYYCNARNLWGQGTLVTVSSDKTHTCPPCPAPESTRGPSVFLFPPKPKDTLMISRTPEVTCVVVDVSHEDPEVKFNWYVDGVEVHNAKTKPREEQYNSTYRVVSVLTVLHQDWLNGKEYKCKVSNKALPAPIEKTISKAKGQPREPQVCTLPPSRDELTKNQVSLSCAVKGFYPSDIAVEWESNGQPENNYKTTPPVLDSDGSFFLVSKLTVDKSRWQQGNVFSCSVMHEALHNHYTQKSLSLSPGK

SEQ ID NO: 10 - protein, 464 aa, synthetic construct
QVQLVESGGGVVQPGGSLRLSCAASGFVLRVNTVSWYRQAPGKQRELVALITSESNEYYDDSVKGRFTISRDNAKNTIYLHMNSLKPEDTGVYFCNFITTWGQGTQVTVSSGGGGSGGGGSGGGGSQVQLVESGGGVVQPGGSLRLSCAASGFVLRVNTVSWYRQAPGKQRELVALITSESNEYYDDSVKGRFTISRDNAKNTIYLHMNSLKPEDTGVYFCNFITTWGQGTQVTVSSDKTHTCPPCPAPESTRGPSVFLFPPKPKDTLMISRTPEVTCVVVDVSHEDPEVKFNWYVDGVEVHNAKTKPREEQYNSTYRVVSVLTVLHQDWLNGKEYKCKVSNKALPAPIEKTISKAKGQPREPQVCTLPPSRDELTKNQVSLSCAVKGFYPSDIAVEWESNGQPENNYKTTPPVLDSDGSFFLVSKLTVDKSRWQQGNVFSCSVMHEALHNHYTQKSLSLSPGK

SEQ ID NO: 11 - protein, 482 aa, synthetic construct
EVQLVESGGGLVQPGGSLRLSCAASGRSFSSFQMGWFRQAPGKEREFVAASGWSGGPTYYWDSVIGRFTISTDNSKNTLYLQMNSLRAEDTAVYYCYEDRVLSGRPVRYWGQGTLVTVSSGGGGSGGGGSGGGGSEVQLVESGGGLVQPGGSLRLSCAASGRSFSSFQMGWFRQAPGKEREFVAASGWSGGPTYYWDSVIGRFTISTDNSKNTLYLQMNSLRAEDTAVYYCYEDRVLSGRPVRYWGQGTLVTVSSDKTHTCPPCPAPESTRGPSVFLFPPKPKDTLMISRTPEVTCVVVDVSHEDPEVKFNWYVDGVEVHNAKTKPREEQYNSTYRVVSVLTVLHQDWLNGKEYKCKVSNKALPAPIEKTISKAKGQPREPQVCTLPPSRDELTKNQVSLSCAVKGFYPSDIAVEWESNGQPENNYKTTPPVLDSDGSFFLVSKLTVDKSRWQQGNVFSCSVMHEALHNHYTQKSLSLSPGK

SEQ ID NO: 12 - protein, 482 aa, synthetic construct
EVQLVESGGGLVQPGGSLRLSCAASGRSFSSFQMGWFRQAPGKEREFVAASGWSGGPTYYWDSVIGRFTISTDNSKNTLYLQMNSLRAEDTAVYYCYEDRVLSGRHVRYWGQGTLVTVSSGGGGSGGGGSGGGGSEVQLVESGGGLVQPGGSLRLSCAASGRSFSSFQMGWFRQAPGKEREFVAASGWSGGPTYYWDSVIGRFTISTDNSKNTLYLQMNSLRAEDTAVYYCYEDRVLSGRHVRYWGQGTLVTVSSDKTHTCPPCPAPESTRGPSVFLFPPKPKDTLMISRTPEVTCVVVDVSHEDPEVKFNWYVDGVEVHNAKTKPREEQYNSTYRVVSVLTVLHQDWLNGKEYKCKVSNKALPAPIEKTISKAKGQPREPQVCTLPPSRDELTKNQVSLSCAVKGFYPSDIAVEWESNGQPENNYKTTPPVLDSDGSFFLVSKLTVDKSRWQQGNVFSCSVMHEALHNHYTQKSLSLSPGK

SEQ ID NO: 13 - protein, 581 aa, synthetic construct
EVQLVESGGGLVQPGGSLRLSCAASGFISRFYAMGWYRQAPGKQRELVARISSMGWTYYADSVKGRFTISIDNSKNTLYLQMNSLRAEDTAVYYCNARNLWGQGTLVTVSSGGGGSGGGGSGGGGSEVQLVESGGGLVQPGRSLRLSCAASGFTFNTYAMNWVRQAPGKGLEWVARIRSKYNNYATYYADSVKDRFTISRDDSKSIAYLQMNSLKTEDTAVYYCVRHGNFGNSYVSWFAYWGQGTLVTVSSASTKGPSVFPLAPSSKSTSGGTAALGCLVKDYFPEPVTVSWNSGALTSGVHTFPAVLQSSGLYSLSSVVTVPSSSLGTQTYICNVNHKPSNTKVDKKVEPKSCDKTHTCPPCPAPESTRGPSVFLFPPKPKDTLMISRTPEVTCVVVDVSHEDPEVKFNWYVDGVEVHNAKTKPREEQYNSTYRVVSVLTVLHQDWLNGKEYKCKVSNKALPAPIEKTISKAKGQPREPQVYTLPPCRDELTKNQVSLWCLVKGFYPSDIAVEWESNGQPENNYKTTPPVLDSDGSFFLYSKLTVDKSRWQQGNVFSCSVMHEALHNHYTQKSLSLSPGK

SEQ ID NO: 14 - protein, 581 aa, synthetic construct
EVQLVESGGGLVQPGGSLRLSCAASYFISRFYAVGWYRQAPGKQRELVARISSGGWTYYADSVKGRFTISIDNSKNTLYLQMNSLRAEDTAVYYCNARNLWGQGTLVTVSSGGGGSGGGGSGGGGSEVQLVESGGGLVQPGRSLRLSCAASGFTFNTYAMNWVRQAPGKGLEWVARIRSKYNNYATYYADSVKDRFTISRDDSKSIAYLQMNSLKTEDTAVYYCVRHGNFGNSYVSWFAYWGQGTLVTVSSASTKGPSVFPLAPSSKSTSGGTAALGCLVKDYFPEPVTVSWNSGALTSGVHTFPAVLQSSGLYSLSSVVTVPSSSLGTQTYICNVNHKPSNTKVDKKVEPKSCDKTHTCPPCPAPESTRGPSVFLFPPKPKDTLMISRTPEVTCVVVDVSHEDPEVKFNWYVDGVEVHNAKTKPREEQYNSTYRVVSVLTVLHQDWLNGKEYKCKVSNKALPAPIEKTISKAKGQPREPQVYTLPPCRDELTKNQVSLWCLVKGFYPSDIAVEWESNGQPENNYKTTPPVLDSDGSFFLYSKLTVDKSRWQQGNVFSCSVMHEALHNHYTQKSLSLSPGK

SEQ ID NO: 15 - protein, 581 aa, synthetic construct
QVQLVESGGGVVQPGGSLRLSCAASGFVLRVNTVSWYRQAPGKQRELVALITSESNEYYDDSVKGRFTISRDNAKNTIYLHMNSLKPEDTGVYFCNFITTWGQGTQVTVSSGGGGSGGGGSGGGGSEVQLVESGGGLVQPGRSLRLSCAASGFTFNTYAMNWVRQAPGKGLEWVARIRSKYNNYATYYADSVKDRFTISRDDSKSIAYLQMNSLKTEDTAVYYCVRHGNFGNSYVSWFAYWGQGTLVTVSSASTKGPSVFPLAPSSKSTSGGTAALGCLVKDYFPEPVTVSWNSGALTSGVHTFPAVLQSSGLYSLSSVVTVPSSSLGTQTYICNVNHKPSNTKVDKKVEPKSCDKTHTCPPCPAPESTRGPSVFLFPPKPKDTLMISRTPEVTCVVVDVSHEDPEVKFNWYVDGVEVHNAKTKPREEQYNSTYRVVSVLTVLHQDWLNGKEYKCKVSNKALPAPIEKTISKAKGQPREPQVYTLPPCRDELTKNQVSLWCLVKGFYPSDIAVEWESNGQPENNYKTTPPVLDSDGSFFLYSKLTVDKSRWQQGNVFSCSVMHEALHNHYTQKSLSLSPGK

SEQ ID NO: 16 - protein, 590 aa, synthetic construct
EVQLVESGGGLVQPGGSLRLSCAASGRSFSSFQMGWFRQAPGKEREFVAASGWSGGPTYYWDSVIGRFTISTDNSKNTLYLQMNSLRAEDTAVYYCYEDRVLSGRPVRYWGQGTLVTVSSGGGGSGGGGSGGGGSEVQLVESGGGLVQPGRSLRLSCAASGFTFNTYAMNWVRQAPGKGLEWVARIRSKYNNYATYYADSVKDRFTISRDDSKSIAYLQMNSLKTEDTAVYYCVRHGNFGNSYVSWFAYWGQGTLVTVSSASTKGPSVFPLAPSSKSTSGGTAALGCLVKDYFPEPVTVSWNSGALTSGVHTFPAVLQSSGLYSLSSVVTVPSSSLGTQTYICNVNHKPSNTKVDKKVEPKSCDKTHTCPPCPAPESTRGPSVFLFPPKPKDTLMISRTPEVTCVVVDVSHEDPEVKFNWYVDGVEVHNAKTKPREEQYNSTYRVVSVLTVLHQDWLNGKEYKCKVSNKALPAPIEKTISKAKGQPREPQVYTLPPCRDELTKNQVSLWCLVKGFYPSDIAVEWESNGQPENNYKTTPPVLDSDGSFFLYSKLTVDKSRWQQGNVFSCSVMHEALHNHYTQKSLSLSPGK

SEQ ID NO: 17 - protein, 590 aa, synthetic construct
EVQLVESGGGLVQPGGSLRLSCAASGRSFSSFQMGWFRQAPGKEREFVAASGWSGGPTYYWDSVIGRFTISTDNSKNTLYLQMNSLRAEDTAVYYCYEDRVLSGRHVRYWGQGTLVTVSSGGGGSGGGGSGGGGSEVQLVESGGGLVQPGRSLRLSCAASGFTFNTYAMNWVRQAPGKGLEWVARIRSKYNNYATYYADSVKDRFTISRDDSKSIAYLQMNSLKTEDTAVYYCVRHGNFGNSYVSWFAYWGQGTLVTVSSASTKGPSVFPLAPSSKSTSGGTAALGCLVKDYFPEPVTVSWNSGALTSGVHTFPAVLQSSGLYSLSSVVTVPSSSLGTQTYICNVNHKPSNTKVDKKVEPKSCDKTHTCPPCPAPESTRGPSVFLFPPKPKDTLMISRTPEVTCVVVDVSHEDPEVKFNWYVDGVEVHNAKTKPREEQYNSTYRVVSVLTVLHQDWLNGKEYKCKVSNKALPAPIEKTISKAKGQPREPQVYTLPPCRDELTKNQVSLWCLVKGFYPSDIAVEWESNGQPENNYKTTPPVLDSDGSFFLYSKLTVDKSRWQQGNVFSCSVMHEALHNHYTQKSLSLSPGK

SEQ ID NO: 18 - protein, 111 aa, synthetic construct
EVQLVESGGGLVQPGGSLRLSCAASGFISRFYAMGWYRQAPGKQRELVARISSMGWTYYADSVKGRFTISIDNSKNTLYLQMNSLRAEDTAVYYCNARNLWGQGTLVTVSS

SEQ ID NO: 19 - protein, 8 aa, synthetic construct
GFISRFYA

SEQ ID NO: 20 - protein, 7 aa, synthetic construct
ISSMGWT

SEQ ID NO: 21 - protein, 5 aa, synthetic construct
NARNL

SEQ ID NO: 22 - protein, 111 aa, synthetic construct
EVQLVESGGGLVQPGGSLRLSCAASYFISRFYAVGWYRQAPGKQRELVARISSGGWTYYADSVKGRFTISIDNSKNTLYLQMNSLRAEDTAVYYCNARNLWGQGTLVTVSS

SEQ ID NO: 23 - protein, 8 aa, synthetic construct
YFISRFYA

SEQ ID NO: 24 - protein, 7 aa, synthetic construct
ISSGGWT

SEQ ID NO: 25 - protein, 5 aa, synthetic construct
NARNL

SEQ ID NO: 26 - protein, 111 aa, synthetic construct
QVQLVESGGGVVQPGGSLRLSCAASGFVLRVNTVSWYRQAPGKQRELVALITSESNEYYDDSVKGRFTISRDNAKNTIYLHMNSLKPEDTGVYFCNFITTWGQGTQVTVSS

SEQ ID NO: 27 - protein, 8 aa, synthetic construct
GFVLRVNT

SEQ ID NO: 28 - protein, 7 aa, synthetic construct
ITSESNE

SEQ ID NO: 29 - protein, 5 aa, synthetic construct
NFITT

SEQ ID NO: 30 - protein, 120 aa, synthetic construct
EVQLVESGGGLVQPGGSLRLSCAASGRSFSSFQMGWFRQAPGKEREFVAASGWSGGPTYYWDSVIGRFTISTDNSKNTLYLQMNSLRAEDTAVYYCYEDRVLSGRPVRYWGQGTLVTVSS

SEQ ID NO: 31 - protein, 8 aa, synthetic construct
GRSFSSFQ

SEQ ID NO: 32 - protein, 8 aa, synthetic construct
SGWSGGPT

SEQ ID NO: 33 - protein, 13 aa, synthetic construct
YEDRVLSGRPVRY

SEQ ID NO: 34 - protein, 120 aa, synthetic construct
EVQLVESGGGLVQPGGSLRLSCAASGRSFSSFQMGWFRQAPGKEREFVAASGWSGGPTYYWDSVIGRFTISTDNSKNTLYLQMNSLRAEDTAVYYCYEDRVLSGRHVRYWGQGTLVTVSS

SEQ ID NO: 35 - protein, 8 aa, synthetic construct
GRSFSSFQ

SEQ ID NO: 36 - protein, 8 aa, synthetic construct
SGWSGGPT

SEQ ID NO: 37 - protein, 13 aa, synthetic construct
YEDRVLSGRHVRY

SEQ ID NO: 38 - protein, 125 aa, synthetic construct
EVQLVESGGGLVQPGRSLRLSCAASGFTFNTYAMNWVRQAPGKGLEWVARIRSKYNNYATYYADSVKDRFTISRDDSKSIAYLQMNSLKTEDTAVYYCVRHGNFGNSYVSWFAYWGQGTLVTVSS

SEQ ID NO: 39 - protein, 10 aa, synthetic construct
GFTFNTYAMN

SEQ ID NO: 40 - protein, 19 aa, synthetic construct
RIRSKYNNYATYYADSVKD

SEQ ID NO: 41 - protein, 14 aa, synthetic construct
HGNFGNSYVSWFAY

SEQ ID NO: 42 - protein, 109 aa, synthetic construct
QTVVTQEPSLTVSPGGTVTLTCRSSTGAVTTSNYANWVQQKPGQAPRGLIGGTNKRAPGVPARFSGSLLGGKAALTLSGVQPEDEAEYFCALWYSNLWVFGGGTKLTVL

SEQ ID NO: 43 - protein, 14 aa, synthetic construct
RSSTGAVTTSNYAN

SEQ ID NO: 44 - protein, 7 aa, synthetic construct
GTNKRAP

SEQ ID NO: 45 - protein, 9 aa, synthetic construct
ALWYSNLWV

SEQ ID NO: 46 - protein, 227 aa, synthetic construct
DKTHTCPPCPAPESTRGPSVFLFPPKPKDTLMISRTPEVTCVVVDVSHEDPEVKFNWYVDGVEVHNAKTKPREEQYNSTYRVVSVLTVLHQDWLNGKEYKCKVSNKALPAPIEKTISKAKGQPREPQVCTLPPSRDELTKNQVSLSCAVKGFYPSDIAVEWESNGQPENNYKTTPPVLDSDGSFFLVSKLTVDKSRWQQGNVFSCSVMHEALHNHYTQKSLSLSPGK

SEQ ID NO: 47 - protein, 106 aa, synthetic construct
GQPKAAPSVTLFPPSSEELQANKATLVCLISDFYPGAVTVAWKADSSPVKAGVETTTPSKQSNNKYAASSYLSLTPEQWKSHRSYSCQVTHEGSTVEKTVAPTECS

SEQ ID NO: 48 - protein, 330 aa, synthetic construct
ASTKGPSVFPLAPSSKSTSGGTAALGCLVKDYFPEPVTVSWNSGALTSGVHTFPAVLQSSGLYSLSSVVTVPSSSLGTQTYICNVNHKPSNTKVDKKVEPKSCDKTHTCPPCPAPESTRGPSVFLFPPKPKDTLMISRTPEVTCVVVDVSHEDPEVKFNWYVDGVEVHNAKTKPREEQYNSTYRVVSVLTVLHQDWLNGKEYKCKVSNKALPAPIEKTISKAKGQPREPQVYTLPPCRDELTKNQVSLWCLVKGFYPSDIAVEWESNGQPENNYKTTPPVLDSDGSFFLYSKLTVDKSRWQQGNVFSCSVMHEALHNHYTQKSLSLSPGK

SEQ ID NO: 49 - protein, 15 aa, synthetic construct
GGGGSGGGGSGGGGS

SEQ ID NO: 50 - protein, 5 aa, synthetic construct
  REGION >5: note = The entire sequence of amino acids 1-5 can be repeated one or more times.; note (original language) = 氨基酸1-5的整个序列可以重复一次或更多次。
GGGGS